European Patent Application EP 4 173 494 A1, published May 3, 2023. Title: COMPOSITION FOR PREVENTING, AMELIORATING, OR TREATING DISEASE CAUSED BY NITRATION OF TYROSINE IN PROTEINS COMPRISING TYROSINE AS EFFECTIVE COMPONENT. Applicant: INDUSTRY-ACADEMIC COOPERATION FOUNDATION GYEONGSANG NATIONAL UNIVERSITY. The sequence listing filed with the application follows.

SEQUENCE LISTING (8 sequences)

SEQ ID NO: 1 - DNA, 23 bp, Artificial Sequence
  IL-1beta f
tcgcagcagcacatcaacaagag

SEQ ID NO: 2 - DNA, 23 bp, Artificial Sequence
  IL-1beta r
ggtgctcatgtcctcatcctgga

SEQ ID NO: 3 - DNA, 20 bp, Artificial Sequence
  IL-6f
ccaattcatcttgaaatcac

SEQ ID NO: 4 - DNA, 20 bp, Artificial Sequence
  IL-6r
ggaatgtccacaaactgata

SEQ ID NO: 5 - DNA, 24 bp, Artificial Sequence
  NQO-1f
atgacatcacaggtgagctgaagg

SEQ ID NO: 6 - DNA, 24 bp, Artificial Sequence
  NQO-1r
ctcaaaccagcctttcagaatggc

SEQ ID NO: 7 - DNA, 21 bp, Artificial Sequence
  GAPDHf
gtggcaaagtggagattgttg

SEQ ID NO: 8 - DNA, 21 bp, Artificial Sequence
  GAPDHr
ttgactgtgccgttgaatttg